European Patent Application EP 4 481 057 A1, published December 25, 2024. Title: SAMPLE PREPARATION METHODS USING MODIFIED BASES FOR RAPID IDENTIFICATION AND SEQUENCING. Applicant: DEPIXUS. The sequence listing filed with the application follows.

SEQUENCE LISTING (23 sequences)

SEQ ID NO: 1 - DNA, 23 bp, synthetic construct
  source 1..23: mol_type = other DNA
cggtggtctcggaattaatggac

SEQ ID NO: 2 - DNA, 200 bp, synthetic construct
  source 1..200: mol_type = other DNA
cggtggtctcgcgcttctctcacgcgttgtcacttcgctggacggctttggactcgggcctacggtctgctactggggctcagcggccctcagggcctcggagcttggcggaggcctggctagctctgtctaggcctgctcatcggctgggatccgtgcctatccctccgtatgctggtccattaattccgagaccaccg

SEQ ID NO: 3 - DNA, 33 bp, synthetic construct
  source 1..33: mol_type = other DNA
ggctcgtctctcctggacaggaacagaggggca

SEQ ID NO: 4 - DNA, 16 bp, synthetic construct
  source 1..16: mol_type = other DNA
tgcccctctgttcctg

SEQ ID NO: 5 - DNA, 200 bp, synthetic construct
  source 1..200: mol_type = other DNA
tatgtacttcgtctcgctccgtcctcgatcctgtcgccccgctgcggtgtctggcacccttgtggacgggtcccggtgctgcccttctgttgatccggtggctatccgctggtactctgtttcatttccctcctcggccgcctttcatgtggggtcccgctcgccgatccgtggtgcggggcttagagacctgcaactgt

SEQ ID NO: 6 - DNA, 200 bp, synthetic construct
  source 1..200: mol_type = other DNA
tatgtacttcgtctcgctcccccggcggatttcctggtcagtggtgccggttccccggtgtcgtcagtgttctctcggtcccctcgcatggtcgccggccgcgagttccgcccggaccgtccgggaggtcgctgttccggcactcgccctccgccgacgctcctgtcggggcccactgtggcttagagacctgcaactgt

SEQ ID NO: 7 - DNA, 200 bp, synthetic construct
  source 1..200: mol_type = other DNA
tatgtacttcgtctcgctccgctccggggatgggggggggccctgccgttgttgctggtgtgtattctggtgtgcgttgttgcgccgtagtcgtcgcgtcccagcctttcggtcccgagtttcgttgatccgtctggcgtttaccgtctgtgttgccttctaccgcttcccctcctgtttgcttagagacctgcaactgt

SEQ ID NO: 8 - DNA, 200 bp, synthetic construct
  source 1..200: mol_type = other DNA
tatgtacttcgtctcgctcccggcaccttcgcccattctgtcctttcctgatgttcgtcttattgttcgggacgccccttccgtggtcgaggccgtccgaggctttgttcgcgttaccgcgttttctccattcctggctcgcttgttgtcggagggtgcggtttttacttcgtcttggtggcttagagacctgcaactgt

SEQ ID NO: 9 - DNA, 200 bp, synthetic construct
  source 1..200: mol_type = other DNA
tatgtacttcgtctcgctccctgtccagcttccgcgatgctcgtgtcgttgaccctccccgtaccctgccttgatctcgcgtgtcggcacgctggcctacgcttttggatcggtgggcctatccctcgcctcttccctcgtccttgcagtccgcgctccgttacggggtgccagccgtttgcttagagacctgcaactgt

SEQ ID NO: 10 - DNA, 505 bp, synthetic construct
  source 1..505: mol_type = other DNA
gccgacgcttgtagtcgcagcctgtcgttagtatcgtagccagatagaaagcttgctgatccgcttaagctagatagactgtttgtctgcacagctccgaagccagaagtaccgatgatcgcctgtataaagtcgcctgtagtcgcttgtaatgtcgttagtaagactgacgtcgtcgaactagtaagaatagaccgaagacgtcctgtaagcaatacgatcacctgccatgcatagatgcttattgtcgatgtcactcgtcagtaagtacgccgcctgtcccgcacagcttagatgccatagttcgacgaatagctcagttgattcacgtcacgaatacgcccagtagtctagaagcctcgacgaaatgctgactgaaagctgaagtctacgtagacagtacttgcaaacgtagaagtcttcgatgaagatctgccgatcgttacgttagatagcccgccatgaagatgaagatgctgtcgacttgtatgtcgctttgcagccg

SEQ ID NO: 11 - DNA, 219 bp, synthetic construct
  source 1..219: mol_type = other DNA
tgtgtcttttggtctttctggtgctcttcgaattttctggtgctcttcatagttgagagtagtttataagaattaaaggataagggatttataagggatatggtatttggttggagtgtgagaaaaagttattagttaagggatagaagttttattggtagatataagaaggtggataaaggtggatcctcttgctgctggtcctgtccgagctagctg

SEQ ID NO: 12 - DNA, 225 bp, synthetic construct
  source 1..225: mol_type = other DNA
tgtgtcttttggtctttctggtgctcttcgaattttctggtgctcttcaagtgtggggaagggggtattatgagagtgaatgaaataagattatgatggaggtgatgtattgttaaggagtcttggttattttatagttgagagtagtttataagaattaaaggataagggatttataagggatatggtatatcctcttgctgctggtcctgtccgagctagctg

SEQ ID NO: 13 - DNA, 267 bp, synthetic construct
  source 1..267: mol_type = other DNA
tgtgtcttttggtctttctggtgctcttcgaattttctggtgctcttctgtctacgtagacttcagctttcagtcagcatttcgtcgaggcttctagactactgggcgtattcgtgacgtgaatcaactgagctattcgtcgaactatggcatctaagctgtgcgggacaggcggcgtacttactgacgagtgacatcgacaataagcatctatgcatggcaggtgatcgtatatcctcttgctgctggtcctgtccgagctagctg

SEQ ID NO: 14 - DNA, 222 bp, synthetic construct
  source 1..222: mol_type = other DNA
tgtgtcttttggtctttctggtgctcttcgaattttctggtgctcttccggtgaaaggaataaagtgaagatttatttatgggggtattaagtaagatggagatttatgaagatttagtttgaagtatgttagtagattcagtttagtagatttgtgaggtttagatatggggtattgtgagtgaataatcctcttgctgctggtcctgtccgagctagctg

SEQ ID NO: 15 - DNA, 26 bp, synthetic construct
  source 1..26: mol_type = other DNA
  modified_base order(14,17): mod_base = OTHER; note = Digoxigenin-X-(5-aminoallyl)-2'-thymidine
gcttgcactgaganttntctcagtgc

SEQ ID NO: 16 - DNA, 52 bp, synthetic construct
  source 1..52: mol_type = other DNA
  modified_base 1: mod_base = OTHER; note = 5-Dibenzylcyclooctyne-2'-deoxyguanosine
ntcgctgcgtagatcgccgagaatcatagatggagtgtggtgtgccttgaaa

SEQ ID NO: 17 - DNA, 62 bp, synthetic construct
  source 1..62: mol_type = other DNA
  modified_base 28: mod_base = OTHER; note = 5-[4-azido-butamido-N-hex-6-yl)-3-acrylimido]-2'-deoxyUridine
tgattctcggcgatctacgcagcgacnatgcagtgtgtcttttggtctttctggtgctcttc

SEQ ID NO: 18 - DNA, 76 bp, synthetic construct
  source 1..76: mol_type = other DNA
attcgaagagcaccagaaagaccaaaagacacaaagggtcagtgctgcaacccacttcctaatctgtcatcttctg

SEQ ID NO: 19 - DNA, 76 bp, synthetic construct
  source 1..76: mol_type = other DNA
ggaggaagagcaccagaaagaccaaaagacacaaagggtcagtgctgcaacccacttcctaatctgtcatcttctg

SEQ ID NO: 20 - DNA, 51 bp, synthetic construct
  source 1..51: mol_type = other DNA
  modified_base order(12,15): mod_base = OTHER; note = Digoxigenin-X-(5-aminoallyl)-2'-thymidine
cgagctagctgnttncagctagctcggaggtcaggcgtgggttggtcctcg

SEQ ID NO: 21 - DNA, 80 bp, synthetic construct
  source 1..80: mol_type = other DNA
  modified_base 27: mod_base = OTHER; note = 5-[4-azido-butamido-N-hex-6-yl)-3-acrylimido]-2'-deoxyUridine
tgattctcggcgatctacgcagcgacngcaagggcgagtgctcttctcatattggcgctaccactccacctcccgctcat

SEQ ID NO: 22 - DNA, 85 bp, synthetic construct
  source 1..85: mol_type = other DNA
tgagcgggaggtggagtggtagcgccaatatgagaagagcgcagggagggaggagtgaacccacttcctaatctgtcatcttctg

SEQ ID NO: 23 - DNA, 20 bp, synthetic construct
  source 1..20: mol_type = other DNA
acagttgcaggtctctaagc